European Patent Application EP 4 549 589 A1, published May 7, 2025. Title: Method of screening stevia plant. Applicant: SUNTORY HOLDINGS LIMITED. The sequence listing filed with the application follows.

SEQUENCE LISTING (54 sequences)

SEQ ID NO: 1 - DNA, 215 bp, Stevia rebaudiana
  source 1..215: mol_type = genomic DNA
aatggcaagcagaaatcgccagcttatagaatcaaatgcctttttaaaatcaaccttaaatagcataagtttatgtttatcttttttggcccaatttacacctcattaatcatgatgtgcccatcaaagatgcttcgaccttgaatgtaggttgattgtttaggaacaattacgttatgaatgatcttttgaatccgaattgccaacaactttcc

SEQ ID NO: 2 - DNA, 204 bp, Stevia rebaudiana
  source 1..204: mol_type = genomic DNA
aaaggacccagtggtggttgttcgtgacggccagaaccccgtcttagggccatagcgacggcggctagggtttacagccgtgaactctggtcccaactcagttcatttgcgattttcggctgaaataggtaagctctgactcccttttgttgcgaaatcgctcccgatcttgcttccttttcctcaatctagcttaatgtcggt

SEQ ID NO: 3 - DNA, 121 bp, Stevia rebaudiana
  source 1..121: mol_type = genomic DNA
tggtcctttgtcatggtcgattctttagtttgcatgattaagtattctcagcaagcagtttttataaaaagtgactggaacaatgtctaactaggggtgatattctagatggtaagtaaca

SEQ ID NO: 4 - DNA, 20 bp, synthetic construct
  misc_feature 1..20: note = Synthetic DNA
  source 1..20: mol_type = other DNA
aatggcaagcagaaatcgcc

SEQ ID NO: 5 - DNA, 22 bp, synthetic construct
  misc_feature 1..22: note = Synthetic DNA
  source 1..22: mol_type = other DNA
ggaaagttgttggcaattcgga

SEQ ID NO: 6 - DNA, 20 bp, synthetic construct
  misc_feature 1..20: note = Synthetic DNA
  source 1..20: mol_type = other DNA
aaaggacccagtggtggttg

SEQ ID NO: 7 - DNA, 25 bp, synthetic construct
  misc_feature 1..25: note = Synthetic DNA
  source 1..25: mol_type = other DNA
accgacattaagctagattgaggaa

SEQ ID NO: 8 - DNA, 21 bp, synthetic construct
  misc_feature 1..21: note = Synthetic DNA
  source 1..21: mol_type = other DNA
tggtcctttgtcatggtcgat

SEQ ID NO: 9 - DNA, 27 bp, synthetic construct
  misc_feature 1..27: note = Synthetic DNA
  source 1..27: mol_type = other DNA
tgttacttaccatctagaatatcaccc

SEQ ID NO: 10 - DNA, 215 bp, Stevia rebaudiana
  source 1..215: mol_type = genomic DNA
aatggcaagcagaaatcgccagcttatagaatcaaatgcctttttaaaatcaaccttaaatagcataagtttatgtttatcttttttggcccaatttacacctcattaatcatgatgtgcccatcaaagatgcttcgaccttgaatgtaggttgattgtttaggaacaattacgttatgaatggtcttttgaatccgaattgccaacaactttcc

SEQ ID NO: 11 - DNA, 21 bp, Stevia rebaudiana
  source 1..21: mol_type = genomic DNA
gttatgaatggtcttttgaat

SEQ ID NO: 12 - DNA, 41 bp, Stevia rebaudiana
  source 1..41: mol_type = genomic DNA
gaacaattacgttatgaatggtcttttgaatccgaattgcc

SEQ ID NO: 13 - DNA, 61 bp, Stevia rebaudiana
  source 1..61: mol_type = genomic DNA
gattgtttaggaacaattacgttatgaatggtcttttgaatccgaattgccaacaactttc

SEQ ID NO: 14 - DNA, 204 bp, Stevia rebaudiana
  source 1..204: mol_type = genomic DNA
aaaggacccagtggtggttgttcgtgacggccagaaccccgtcttagggccatagcgacggcggctagggtttacagccgtgaactctggtcccaactcagttcatttgcgattttcggctgaaataggtaagctctgactcccttttgttgcgaaatcgctcccgatcctgcttccttttcctcaatctagcttaatgtcggt

SEQ ID NO: 15 - DNA, 21 bp, Stevia rebaudiana
  source 1..21: mol_type = genomic DNA
gctcccgatcctgcttccttt

SEQ ID NO: 16 - DNA, 41 bp, Stevia rebaudiana
  source 1..41: mol_type = genomic DNA
ttgcgaaatcgctcccgatcctgcttccttttcctcaatct

SEQ ID NO: 17 - DNA, 61 bp, Stevia rebaudiana
  source 1..61: mol_type = genomic DNA
ctcccttttgttgcgaaatcgctcccgatcctgcttccttttcctcaatctagcttaatgt

SEQ ID NO: 18 - DNA, 121 bp, Stevia rebaudiana
  source 1..121: mol_type = genomic DNA
tggtcctttgtcatggtcgattctttagtttgcatgattaagtattctcagcaagcagtttttataaaaagtgactggaacaatgtctaaccaggggtgatattctagatggtaagtaaca

SEQ ID NO: 19 - DNA, 21 bp, Stevia rebaudiana
  source 1..21: mol_type = genomic DNA
aatgtctaaccaggggtgata

SEQ ID NO: 20 - DNA, 41 bp, Stevia rebaudiana
  source 1..41: mol_type = genomic DNA
tgactggaacaatgtctaaccaggggtgatattctagatgg

SEQ ID NO: 21 - DNA, 61 bp, Stevia rebaudiana
  source 1..61: mol_type = genomic DNA
ttataaaaagtgactggaacaatgtctaaccaggggtgatattctagatggtaagtaacat

SEQ ID NO: 22 - DNA, 20 bp, synthetic construct
  misc_feature 1..20: note = Synthetic DNA
  source 1..20: mol_type = other DNA
attttcttccaaaccccttt

SEQ ID NO: 23 - DNA, 36 bp, synthetic construct
  misc_feature 1..36: note = Synthetic DNA
  source 1..36: mol_type = other DNA
ttattggaaagttgttggcaattcggattcaagata

SEQ ID NO: 24 - DNA, 248 bp, synthetic construct
  misc_feature 1..248: note = Synthetic DNA
  source 1..248: mol_type = other DNA
attttcttccaaaccccttttgatccataatggcaagcagaaatcgccagcttatagaatcaaatgcctttttaaaatcaaccttaaatagcataagtttatgtttatcttttttggcccaatttacacctcattaatcatgatgtgcccatcaaagatgcttcgaccttgaatgtaggttgattgtttaggaacaattacgttatgaatgatatcttgaatccgaattgccaacaactttccaataa

SEQ ID NO: 25 - DNA, 248 bp, synthetic construct
  misc_feature 1..248: note = Synthetic DNA
  source 1..248: mol_type = other DNA
attttcttccaaaccccttttgatccataatggcaagcagaaatcgccagcttatagaatcaaatgcctttttaaaatcaaccttaaatagcataagtttatgtttatcttttttggcccaatttacacctcattaatcatgatgtgcccatcaaagatgcttcgaccttgaatgtaggttgattgtttaggaacaattacgttatgaatggtatcttgaatccgaattgccaacaactttccaataa

SEQ ID NO: 26 - DNA, 213 bp, synthetic construct
  misc_feature 1..213: note = Synthetic DNA
  source 1..213: mol_type = other DNA
attttcttccaaaccccttttgatccataatggcaagcagaaatcgccagcttatagaatcaaatgcctttttaaaatcaaccttaaatagcataagtttatgtttatcttttttggcccaatttacacctcattaatcatgatgtgcccatcaaagatgcttcgaccttgaatgtaggttgattgtttaggaacaattacgttatgaatgat

SEQ ID NO: 27 - DNA, 35 bp, synthetic construct
  misc_feature 1..35: note = Synthetic DNA
  source 1..35: mol_type = other DNA
atcttgaatccgaattgccaacaactttccaataa

SEQ ID NO: 28 - DNA, 20 bp, synthetic construct
  misc_feature 1..20: note = Synthetic DNA
  source 1..20: mol_type = other DNA
gagcctcctgttactgattg

SEQ ID NO: 29 - DNA, 37 bp, synthetic construct
  misc_feature 1..37: note = Synthetic DNA
  source 1..37: mol_type = other DNA
tataccgacattaagctagattgaggaaaaggcagct

SEQ ID NO: 30 - DNA, 242 bp, synthetic construct
  misc_feature 1..242: note = Synthetic DNA
  source 1..242: mol_type = other DNA
gagcctcctgttactgattggggctcagtttgagtaaaggacccagtggtggttgttcgtgacggccagaaccccgtcttagggccatagcgacggcggctagggtttacagccgtgaactctggtcccaactcagttcatttgcgattttcggctgaaataggtaagctctgactcccttttgttgcgaaatcgctcccgatctagctgccttttcctcaatctagcttaatgtcggtata

SEQ ID NO: 31 - DNA, 242 bp, synthetic construct
  misc_feature 1..242: note = Synthetic DNA
  source 1..242: mol_type = other DNA
gagcctcctgttactgattggggctcagtttgagtaaaggacccagtggtggttgttcgtgacggccagaaccccgtcttagggccatagcgacggcggctagggtttacagccgtgaactctggtcccaactcagttcatttgcgattttcggctgaaataggtaagctctgactcccttttgttgcgaaatcgctcccgatccagctgccttttcctcaatctagcttaatgtcggtata

SEQ ID NO: 32 - DNA, 207 bp, synthetic construct
  misc_feature 1..207: note = Synthetic DNA
  source 1..207: mol_type = other DNA
gagcctcctgttactgattggggctcagtttgagtaaaggacccagtggtggttgttcgtgacggccagaaccccgtcttagggccatagcgacggcggctagggtttacagccgtgaactctggtcccaactcagttcatttgcgattttcggctgaaataggtaagctctgactcccttttgttgcgaaatcgctcccgatccag

SEQ ID NO: 33 - DNA, 35 bp, synthetic construct
  misc_feature 1..35: note = Synthetic DNA
  source 1..35: mol_type = other DNA
ctgccttttcctcaatctagcttaatgtcggtata

SEQ ID NO: 34 - DNA, 19 bp, synthetic construct
  misc_feature 1..19: note = Synthetic DNA
  source 1..19: mol_type = other DNA
ggatggggaatagatgaac

SEQ ID NO: 35 - DNA, 37 bp, synthetic construct
  misc_feature 1..37: note = Synthetic DNA
  source 1..37: mol_type = other DNA
tgcatatatgttacttaccatctagaatatcacagct

SEQ ID NO: 36 - DNA, 284 bp, synthetic construct
  misc_feature 1..284: note = Synthetic DNA
  source 1..284: mol_type = other DNA
ggatggggaatagatgaacaaagttaatgtaaaaagctaaattttaagcaactttgaaatttttggaaaatgccttaaggcgagttcaaatgcagttaaaagtcagatttttcagtttaaatcaccaacttcttacctgctagcgaattggtttttggtcctttgtcatggtcgattctttagtttgcatgattaagtattctcagcaagcagtttttataaaaagtgactggaacaatgtctaaccagctgtgatattctagatggtaagtaacatatatgca

SEQ ID NO: 37 - DNA, 249 bp, synthetic construct
  misc_feature 1..249: note = Synthetic DNA
  source 1..249: mol_type = other DNA
ggatggggaatagatgaacaaagttaatgtaaaaagctaaattttaagcaactttgaaatttttggaaaatgccttaaggcgagttcaaatgcagttaaaagtcagatttttcagtttaaatcaccaacttcttacctgctagcgaattggtttttggtcctttgtcatggtcgattctttagtttgcatgattaagtattctcagcaagcagtttttataaaaagtgactggaacaatgtctaaccag

SEQ ID NO: 38 - DNA, 35 bp, synthetic construct
  misc_feature 1..35: note = Synthetic DNA
  source 1..35: mol_type = other DNA
ctgtgatattctagatggtaagtaacatatatgca

SEQ ID NO: 39 - DNA, 284 bp, synthetic construct
  misc_feature 1..284: note = Synthetic DNA
  source 1..284: mol_type = other DNA
ggatggggaatagatgaacaaagttaatgtaaaaagctaaattttaagcaactttgaaatttttggaaaatgccttaaggcgagttcaaatgcagttaaaagtcagatttttcagtttaaatcaccaacttcttacctgctagcgaattggtttttggtcctttgtcatggtcgattctttagtttgcatgattaagtattctcagcaagcagtttttataaaaagtgactggaacaatgtctaactagctgtgatattctagatggtaagtaacatatatgca

SEQ ID NO: 40 - DNA, 21 bp, Stevia rebaudiana
  source 1..21: mol_type = genomic DNA
gttatgaatgatcttttgaat

SEQ ID NO: 41 - DNA, 41 bp, Stevia rebaudiana
  source 1..41: mol_type = genomic DNA
gaacaattacgttatgaatgatcttttgaatccgaattgcc

SEQ ID NO: 42 - DNA, 61 bp, Stevia rebaudiana
  source 1..61: mol_type = genomic DNA
gattgtttaggaacaattacgttatgaatgatcttttgaatccgaattgccaacaactttc

SEQ ID NO: 43 - DNA, 21 bp, Stevia rebaudiana
  source 1..21: mol_type = genomic DNA
gctcccgatcttgcttccttt

SEQ ID NO: 44 - DNA, 41 bp, Stevia rebaudiana
  source 1..41: mol_type = genomic DNA
ttgcgaaatcgctcccgatcttgcttccttttcctcaatct

SEQ ID NO: 45 - DNA, 61 bp, Stevia rebaudiana
  source 1..61: mol_type = genomic DNA
ctcccttttgttgcgaaatcgctcccgatcttgcttccttttcctcaatctagcttaatgt

SEQ ID NO: 46 - DNA, 21 bp, Stevia rebaudiana
  source 1..21: mol_type = genomic DNA
aatgtctaactaggggtgata

SEQ ID NO: 47 - DNA, 41 bp, Stevia rebaudiana
  source 1..41: mol_type = genomic DNA
tgactggaacaatgtctaactaggggtgatattctagatgg

SEQ ID NO: 48 - DNA, 61 bp, Stevia rebaudiana
  source 1..61: mol_type = genomic DNA
ttataaaaagtgactggaacaatgtctaactaggggtgatattctagatggtaagtaacat

SEQ ID NO: 49 - DNA, 248 bp, Stevia rebaudiana
  source 1..248: mol_type = genomic DNA
attttcttccaaaccccttttgatccataatggcaagcagaaatcgccagcttatagaatcaaatgcctttttaaaatcaaccttaaatagcataagtttatgtttatcttttttggcccaatttacacctcattaatcatgatgtgcccatcaaagatgcttcgaccttgaatgtaggttgattgtttaggaacaattacgttatgaatgatcttttgaatccgaattgccaacaactttccaataa

SEQ ID NO: 50 - DNA, 248 bp, Stevia rebaudiana
  source 1..248: mol_type = genomic DNA
attttcttccaaaccccttttgatccataatggcaagcagaaatcgccagcttatagaatcaaatgcctttttaaaatcaaccttaaatagcataagtttatgtttatcttttttggcccaatttacacctcattaatcatgatgtgcccatcaaagatgcttcgaccttgaatgtaggttgattgtttaggaacaattacgttatgaatggtcttttgaatccgaattgccaacaactttccaataa

SEQ ID NO: 51 - DNA, 242 bp, Stevia rebaudiana
  source 1..242: mol_type = genomic DNA
gagcctcctgttactgattggggctcagtttgagtaaaggacccagtggtggttgttcgtgacggccagaaccccgtcttagggccatagcgacggcggctagggtttacagccgtgaactctggtcccaactcagttcatttgcgattttcggctgaaataggtaagctctgactcccttttgttgcgaaatcgctcccgatcttgcttccttttcctcaatctagcttaatgtcggtata

SEQ ID NO: 52 - DNA, 242 bp, Stevia rebaudiana
  source 1..242: mol_type = genomic DNA
gagcctcctgttactgattggggctcagtttgagtaaaggacccagtggtggttgttcgtgacggccagaaccccgtcttagggccatagcgacggcggctagggtttacagccgtgaactctggtcccaactcagttcatttgcgattttcggctgaaataggtaagctctgactcccttttgttgcgaaatcgctcccgatcctgcttccttttcctcaatctagcttaatgtcggtata

SEQ ID NO: 53 - DNA, 284 bp, Stevia rebaudiana
  source 1..284: mol_type = genomic DNA
ggatggggaatagatgaacaaagttaatgtaaaaagctaaattttaagcaactttgaaatttttggaaaatgccttaaggcgagttcaaatgcagttaaaagtcagatttttcagtttaaatcaccaacttcttacctgctagcgaattggtttttggtcctttgtcatggtcgattctttagtttgcatgattaagtattctcagcaagcagtttttataaaaagtgactggaacaatgtctaactaggggtgatattctagatggtaagtaacatatatgca

SEQ ID NO: 54 - DNA, 284 bp, Stevia rebaudiana
  source 1..284: mol_type = genomic DNA
ggatggggaatagatgaacaaagttaatgtaaaaagctaaattttaagcaactttgaaatttttggaaaatgccttaaggcgagttcaaatgcagttaaaagtcagatttttcagtttaaatcaccaacttcttacctgctagcgaattggtttttggtcctttgtcatggtcgattctttagtttgcatgattaagtattctcagcaagcagtttttataaaaagtgactggaacaatgtctaaccaggggtgatattctagatggtaagtaacatatatgca